European Patent Specification EP 3 569 703 B1, published September 23, 2026. Title: 胃蛋白抗性和耐酸性改良及催化效率提高的植酸酶YeAPPA突变体. Applicant: 中国农业科学院饲料研究所. The sequence listing filed with the application follows.

SEQUENCE LISTING (12 sequences)

SEQ ID NO: 1 - protein, 441 aa, Yersinia enterocolitica）
MSVAKRNLHLSALTLIMGCFTAGAAPIATPPASYTLERVVILSRHGVRSPTKQTQLMNDVTPDKWPLWPVKAGYLTPRRAELVTLMGGFYGDYFRSQGLLSAGCPVDGSVYAQADVDQRTRLTGQAFLDGIAPDCGLKVHYQADLKKVDPLFHTVEAGVCKLDSAKTHQAVEERLGGPLSDLSQRYAKPFAQMGEVLNFAASPYCKSLQKNGKTCDFATFTANEIKVNEEGTKVSLSGPLALSSTLGEIFLLQDSQAMPDVAWHRLSGEENWVSLLSLRNAQFDLMAKTPYIARHKGTPLLQQIDTALVLQRDAQGQTLPLSPQTKLLFLGGHDTNIANIAGMLGANWQLPQQPDNTPPGGGLVFELWQNPDNHQRYVAVKMFYQTMDQLRNAEKLDMKNNPAKIVPITIEGCENEGDNKLCQLETFQKKVAQVIEPACHI

SEQ ID NO: 2 - DNA, 1326 bp, Yersinia enterocolitica）
atgtcagttgcaaagagaaatctgcacttatccgcactcactttgataatgggctgttttaccgcaggtgctgccccgattgctacaccgccggccagctacacattagagcgtgtggttattttgagtcgacatggtgttcgctccccgacaaaacaaacccagctaatgaatgatgtcacacctgataaatggcccctgtggccagtaaaagcgggctatttaacaccgcgaagggctgagttagtgactttgatggggggattttatggtgattatttccgcagccaagggttgttgtctgcggggtgtccggtagatggctccgtttatgcacaggcagatgttgaccaacgaacccgcttaaccggacaggcattcttggatgggatcgcaccggattgtggtctgaaagtacattatcaggctgatttgaagaaagttgacccgctatttcataccgtcgaagcgggggtctgtaaactggactcagcgaaaactcatcaggctgttgaggagcgattgggcgggccattgagtgatcttagccagcgctatgccaaaccctttgctcagatgggcgaagtgctgaattttgcagcatcgccttattgcaagtcattgcaaaaaaatggaaaaacctgtgattttgcaacttttacggcaaatgaaattaaggtaaacgaagaaggtactaaagtttctctgagtgggccattggcactatcgtcgacattgggtgaaattttcctgttacaagactcacaagctatgccggatgtggcctggcatcggctcagcggtgaagagaactgggtttcgctattgtcgttgcgcaatgcgcaatttgatttgatggccaaaaccccgtatatcgctcgccataaagggaccccgctgttgcaacaaattgatacggcattagtgctgcaacgcgatgcccaagggcaaacactgccgctgtcaccgcaaaccaaattgctgttcctcggcgggcatgacaccaatattgctaatatcgctggtatgttaggggccaattggcaattaccacagcaacctgataataccccgcctggtggcggattagtctttgagctatggcagaacccagataatcatcagcgctatgtcgccgtgaaaatgttctatcaaacgatggatcagctgcgaaatgccgagaaattagatatgaaaaacaacccagctaaaattgttccaattaccattgaaggttgtgagaacgagggtgataacaaactttgccaacttgagactttccaaaagaaagttgcccaagtgatcgagccagcctgccatatttaa

SEQ ID NO: 3 - protein, 441 aa, 人工序列(Artificial Sequence)
MSVAKRNLHLSALTLIMGCFTAGAAPIATPPASYTLERVVILSRHGVRSPTKQTQLMNDVTPDKWPLWPVKAGYLTPRRAELVTLMGGFYGDYFRSQGLLSAGCPVDGSVYAQADVDQRTRLTGQAFLDGIAPDCGLKVHYQADLKKVDPLFHTVEAGVCKGDSAKTHQAVEERLGGPLSDLSQRYAKPFAQMGEVLNFAASPYCKSLQKNGKTCDFATFTANEIKVNEEGTKVSLSGPLALSSTLGEIFLLQDSQAMPDVAWHRLSGEENWVSLLSLRNAQFDLMAKTPYIARHKGTPLLQQIDTALVLQRDAQGQTLPLSPQTKLLFLGGHDTNIANIAGMLGANWQLPQQPDNTPPGGGLVFELWQNPDNHQRYVAVKMFYQTMDQLRNAEKLDMKNNPAKIVPITIEGCENEGDNKLCQLETFQKKVAQVIEPACHI

SEQ ID NO: 4 - protein, 441 aa, 人工序列(Artificial Sequence)
MSVAKRNLHLSALTLIMGCFTAGAAPIATPPASYTLERVVILSRHGVRSPTKQTQLMNDVTPDKWPLWPVKAGYLTPRRAELVTLMGGFYGDYFRSQGLLSAGCPVDGSVYAQADVDQRTRLTGQAFLDGIAPDCGLKVHYQADLKKVDPLFHTVEAGVCKADSAKTHQAVEERLGGPLSDLSQRYAKPFAQMGEVLNFAASPYCKSLQKNGKTCDFATFTANEIKVNEEGTKVSLSGPLALSSTLGEIFLLQDSQAMPDVAWHRLSGEENWVSLLSLRNAQFDLMAKTPYIARHKGTPLLQQIDTALVLQRDAQGQTLPLSPQTKLLFLGGHDTNIANIAGMLGANWQLPQQPDNTPPGGGLVFELWQNPDNHQRYVAVKMFYQTMDQLRNAEKLDMKNNPAKIVPITIEGCENEGDNKLCQLETFQKKVAQVIEPACHI

SEQ ID NO: 5 - protein, 441 aa, 人工序列(Artificial Sequence)
MSVAKRNLHLSALTLIMGCFTAGAAPIATPPASYTLERVVILSRHGVRSPTKQTQLMNDVTPDKWPLWPVKAGYLTPRRAELVTLMGGFYGDYFRSQGLLSAGCPVDGSVYAQADVDQRTRLTGQAFLDGIAPDCGLKVHYQADLKKVDPLFHTVEAGVCKLDSAKTHQAVEERLGGPLSDLSQRYAKPFAQMGEVLNFAASPYCKSLQKNGKTCDFATFTANEIKVNEGGTKVSLSGPLALSSTLGEIFLLQDSQAMPDVAWHRLSGEENWVSLLSLRNAQFDLMAKTPYIARHKGTPLLQQIDTALVLQRDAQGQTLPLSPQTKLLFLGGHDTNIANIAGMLGANWQLPQQPDNTPPGGGLVFELWQNPDNHQRYVAVKMFYQTMDQLRNAEKLDMKNNPAKIVPITIEGCENEGDNKLCQLETFQKKVAQVIEPACHI

SEQ ID NO: 6 - protein, 441 aa, 人工序列(Artificial Sequence)
MSVAKRNLHLSALTLIMGCFTAGAAPIATPPASYTLERVVILSRHGVRSPTKQTQLMNDVTPDKWPLWPVKAGYLTPRRAELVTLMGGFYGDYFRSQGLLSAGCPVDGSVYAQADVDQRTRLTGQAFLDGIAPDCGLKVHYQADLKKVDPLFHTVEAGVCKLDSAKTHQAVEERLGGPLSDLSQRYAKPFAQMGEVLNFAASPYCKSLQKNGKTCDFATFTANEIKVNEPGTKVSLSGPLALSSTLGEIFLLQDSQAMPDVAWHRLSGEENWVSLLSLRNAQFDLMAKTPYIARHKGTPLLQQIDTALVLQRDAQGQTLPLSPQTKLLFLGGHDTNIANIAGMLGANWQLPQQPDNTPPGGGLVFELWQNPDNHQRYVAVKMFYQTMDQLRNAEKLDMKNNPAKIVPITIEGCENEGDNKLCQLETFQKKVAQVIEPACHI

SEQ ID NO: 7 - protein, 441 aa, 人工序列(Artificial Sequence)
MSVAKRNLHLSALTLIMGCFTAGAAPIATPPASYTLERVVILSRHGVRSPTKQTQLMNDVTPDKWPLWPVKAGYLTPRRAELVTLMGGFYGDYFRSQGLLSAGCPVDGSVYAQADVDQRTRLTGQAFLDGIAPDCGLKVHYQADLKKVDPLFHTVEAGVCKLDSAKTHQAVEERLGGPLSDLSQRYAKPFAQMGEVLNFAASPYCKSLQKNGKTCDFATFTANEIKVNERGTKVSLSGPLALSSTLGEIFLLQDSQAMPDVAWHRLSGEENWVSLLSLRNAQFDLMAKTPYIARHKGTPLLQQIDTALVLQRDAQGQTLPLSPQTKLLFLGGHDTNIANIAGMLGANWQLPQQPDNTPPGGGLVFELWQNPDNHQRYVAVKMFYQTMDQLRNAEKLDMKNNPAKIVPITIEGCENEGDNKLCQLETFQKKVAQVIEPACHI

SEQ ID NO: 8 - DNA, 1326 bp, 人工序列(Artificial Sequence)
atgtcagttgcaaagagaaatctgcacttatccgcactcactttgataatgggctgttttaccgcaggtgctgccccgattgctacaccgccggccagctacacattagagcgtgtggttattttgagtcgacatggtgttcgctccccgacaaaacaaacccagctaatgaatgatgtcacacctgataaatggcccctgtggccagtaaaagcgggctatttaacaccgcgaagggctgagttagtgactttgatggggggattttatggtgattatttccgcagccaagggttgttgtctgcggggtgtccggtagatggctccgtttatgcacaggcagatgttgaccaacgaacccgcttaaccggacaggcattcttggatgggatcgcaccggattgtggtctgaaagtacattatcaggctgatttgaagaaagttgacccgctatttcataccgtcgaagcgggggtctgtaaaggcgactcagcgaaaactcatcaggctgttgaggagcgattgggcgggccattgagtgatcttagccagcgctatgccaaaccctttgctcagatgggcgaagtgctgaattttgcagcatcgccttattgcaagtcattgcaaaaaaatggaaaaacctgtgattttgcaacttttacggcaaatgaaattaaggtaaacgaagaaggtactaaagtttctctgagtgggccattggcactatcgtcgacattgggtgaaattttcctgttacaagactcacaagctatgccggatgtggcctggcatcggctcagcggtgaagagaactgggtttcgctattgtcgttgcgcaatgcgcaatttgatttgatggccaaaaccccgtatatcgctcgccataaagggaccccgctgttgcaacaaattgatacggcattagtgctgcaacgcgatgcccaagggcaaacactgccgctgtcaccgcaaaccaaattgctgttcctcggcgggcatgacaccaatattgctaatatcgctggtatgttaggggccaattggcaattaccacagcaacctgataataccccgcctggtggcggattagtctttgagctatggcagaacccagataatcatcagcgctatgtcgccgtgaaaatgttctatcaaacgatggatcagctgcgaaatgccgagaaattagatatgaaaaacaacccagctaaaattgttccaattaccattgaaggttgtgagaacgagggtgataacaaactttgccaacttgagactttccaaaagaaagttgcccaagtgatcgagccagcctgccatatttaa

SEQ ID NO: 9 - DNA, 1326 bp, 人工序列(Artificial Sequence)
atgtcagttgcaaagagaaatctgcacttatccgcactcactttgataatgggctgttttaccgcaggtgctgccccgattgctacaccgccggccagctacacattagagcgtgtggttattttgagtcgacatggtgttcgctccccgacaaaacaaacccagctaatgaatgatgtcacacctgataaatggcccctgtggccagtaaaagcgggctatttaacaccgcgaagggctgagttagtgactttgatggggggattttatggtgattatttccgcagccaagggttgttgtctgcggggtgtccggtagatggctccgtttatgcacaggcagatgttgaccaacgaacccgcttaaccggacaggcattcttggatgggatcgcaccggattgtggtctgaaagtacattatcaggctgatttgaagaaagttgacccgctatttcataccgtcgaagcgggggtctgtaaagcggactcagcgaaaactcatcaggctgttgaggagcgattgggcgggccattgagtgatcttagccagcgctatgccaaaccctttgctcagatgggcgaagtgctgaattttgcagcatcgccttattgcaagtcattgcaaaaaaatggaaaaacctgtgattttgcaacttttacggcaaatgaaattaaggtaaacgaagaaggtactaaagtttctctgagtgggccattggcactatcgtcgacattgggtgaaattttcctgttacaagactcacaagctatgccggatgtggcctggcatcggctcagcggtgaagagaactgggtttcgctattgtcgttgcgcaatgcgcaatttgatttgatggccaaaaccccgtatatcgctcgccataaagggaccccgctgttgcaacaaattgatacggcattagtgctgcaacgcgatgcccaagggcaaacactgccgctgtcaccgcaaaccaaattgctgttcctcggcgggcatgacaccaatattgctaatatcgctggtatgttaggggccaattggcaattaccacagcaacctgataataccccgcctggtggcggattagtctttgagctatggcagaacccagataatcatcagcgctatgtcgccgtgaaaatgttctatcaaacgatggatcagctgcgaaatgccgagaaattagatatgaaaaacaacccagctaaaattgttccaattaccattgaaggttgtgagaacgagggtgataacaaactttgccaacttgagactttccaaaagaaagttgcccaagtgatcgagccagcctgccatatttaa

SEQ ID NO: 10 - DNA, 1326 bp, 人工序列(Artificial Sequence)
atgtcagttgcaaagagaaatctgcacttatccgcactcactttgataatgggctgttttaccgcaggtgctgccccgattgctacaccgccggccagctacacattagagcgtgtggttattttgagtcgacatggtgttcgctccccgacaaaacaaacccagctaatgaatgatgtcacacctgataaatggcccctgtggccagtaaaagcgggctatttaacaccgcgaagggctgagttagtgactttgatggggggattttatggtgattatttccgcagccaagggttgttgtctgcggggtgtccggtagatggctccgtttatgcacaggcagatgttgaccaacgaacccgcttaaccggacaggcattcttggatgggatcgcaccggattgtggtctgaaagtacattatcaggctgatttgaagaaagttgacccgctatttcataccgtcgaagcgggggtctgtaaactggactcagcgaaaactcatcaggctgttgaggagcgattgggcgggccattgagtgatcttagccagcgctatgccaaaccctttgctcagatgggcgaagtgctgaattttgcagcatcgccttattgcaagtcattgcaaaaaaatggaaaaacctgtgattttgcaacttttacggcaaatgaaattaaggtaaacgaaggcggtactaaagtttctctgagtgggccattggcactatcgtcgacattgggtgaaattttcctgttacaagactcacaagctatgccggatgtggcctggcatcggctcagcggtgaagagaactgggtttcgctattgtcgttgcgcaatgcgcaatttgatttgatggccaaaaccccgtatatcgctcgccataaagggaccccgctgttgcaacaaattgatacggcattagtgctgcaacgcgatgcccaagggcaaacactgccgctgtcaccgcaaaccaaattgctgttcctcggcgggcatgacaccaatattgctaatatcgctggtatgttaggggccaattggcaattaccacagcaacctgataataccccgcctggtggcggattagtctttgagctatggcagaacccagataatcatcagcgctatgtcgccgtgaaaatgttctatcaaacgatggatcagctgcgaaatgccgagaaattagatatgaaaaacaacccagctaaaattgttccaattaccattgaaggttgtgagaacgagggtgataacaaactttgccaacttgagactttccaaaagaaagttgcccaagtgatcgagccagcctgccatatttaa

SEQ ID NO: 11 - DNA, 1326 bp, 人工序列(Artificial Sequence)
atgtcagttgcaaagagaaatctgcacttatccgcactcactttgataatgggctgttttaccgcaggtgctgccccgattgctacaccgccggccagctacacattagagcgtgtggttattttgagtcgacatggtgttcgctccccgacaaaacaaacccagctaatgaatgatgtcacacctgataaatggcccctgtggccagtaaaagcgggctatttaacaccgcgaagggctgagttagtgactttgatggggggattttatggtgattatttccgcagccaagggttgttgtctgcggggtgtccggtagatggctccgtttatgcacaggcagatgttgaccaacgaacccgcttaaccggacaggcattcttggatgggatcgcaccggattgtggtctgaaagtacattatcaggctgatttgaagaaagttgacccgctatttcataccgtcgaagcgggggtctgtaaactggactcagcgaaaactcatcaggctgttgaggagcgattgggcgggccattgagtgatcttagccagcgctatgccaaaccctttgctcagatgggcgaagtgctgaattttgcagcatcgccttattgcaagtcattgcaaaaaaatggaaaaacctgtgattttgcaacttttacggcaaatgaaattaaggtaaacgaaccgggtactaaagtttctctgagtgggccattggcactatcgtcgacattgggtgaaattttcctgttacaagactcacaagctatgccggatgtggcctggcatcggctcagcggtgaagagaactgggtttcgctattgtcgttgcgcaatgcgcaatttgatttgatggccaaaaccccgtatatcgctcgccataaagggaccccgctgttgcaacaaattgatacggcattagtgctgcaacgcgatgcccaagggcaaacactgccgctgtcaccgcaaaccaaattgctgttcctcggcgggcatgacaccaatattgctaatatcgctggtatgttaggggccaattggcaattaccacagcaacctgataataccccgcctggtggcggattagtctttgagctatggcagaacccagataatcatcagcgctatgtcgccgtgaaaatgttctatcaaacgatggatcagctgcgaaatgccgagaaattagatatgaaaaacaacccagctaaaattgttccaattaccattgaaggttgtgagaacgagggtgataacaaactttgccaacttgagactttccaaaagaaagttgcccaagtgatcgagccagcctgccatatttaa

SEQ ID NO: 12 - DNA, 1326 bp, 人工序列(Artificial Sequence)
atgtcagttgcaaagagaaatctgcacttatccgcactcactttgataatgggctgttttaccgcaggtgctgccccgattgctacaccgccggccagctacacattagagcgtgtggttattttgagtcgacatggtgttcgctccccgacaaaacaaacccagctaatgaatgatgtcacacctgataaatggcccctgtggccagtaaaagcgggctatttaacaccgcgaagggctgagttagtgactttgatggggggattttatggtgattatttccgcagccaagggttgttgtctgcggggtgtccggtagatggctccgtttatgcacaggcagatgttgaccaacgaacccgcttaaccggacaggcattcttggatgggatcgcaccggattgtggtctgaaagtacattatcaggctgatttgaagaaagttgacccgctatttcataccgtcgaagcgggggtctgtaaactggactcagcgaaaactcatcaggctgttgaggagcgattgggcgggccattgagtgatcttagccagcgctatgccaaaccctttgctcagatgggcgaagtgctgaattttgcagcatcgccttattgcaagtcattgcaaaaaaatggaaaaacctgtgattttgcaacttttacggcaaatgaaattaaggtaaacgaacgtggtactaaagtttctctgagtgggccattggcactatcgtcgacattgggtgaaattttcctgttacaagactcacaagctatgccggatgtggcctggcatcggctcagcggtgaagagaactgggtttcgctattgtcgttgcgcaatgcgcaatttgatttgatggccaaaaccccgtatatcgctcgccataaagggaccccgctgttgcaacaaattgatacggcattagtgctgcaacgcgatgcccaagggcaaacactgccgctgtcaccgcaaaccaaattgctgttcctcggcgggcatgacaccaatattgctaatatcgctggtatgttaggggccaattggcaattaccacagcaacctgataataccccgcctggtggcggattagtctttgagctatggcagaacccagataatcatcagcgctatgtcgccgtgaaaatgttctatcaaacgatggatcagctgcgaaatgccgagaaattagatatgaaaaacaacccagctaaaattgttccaattaccattgaaggttgtgagaacgagggtgataacaaactttgccaacttgagactttccaaaagaaagttgcccaagtgatcgagccagcctgccatatttaa